European Patent Application EP 4 789 666 A1, published August 12, 2026. Title: RNA M6A REGULATOR COMPOSITION, PREPARATION METHOD THEREFOR, AND USE THEREOF. Applicant: SHANGHAI MERNA THERAPEUTICS CO. LTD. Application EP. The sequence listing filed with the application follows.

SEQUENCE LISTING (8 sequences)

SEQ ID NO: 1 - DNA, 20 bp, synthetic construct
  source 1..20: mol_type = other DNA
gtcaagtcctctggtggcag

SEQ ID NO: 2 - DNA, 20 bp, synthetic construct
  source 1..20: mol_type = other DNA
aaggctgggacaaatcgacc

SEQ ID NO: 3 - DNA, 20 bp, synthetic construct
  source 1..20: mol_type = other DNA
cccgggtgttgatctgactc

SEQ ID NO: 4 - DNA, 20 bp, synthetic construct
  source 1..20: mol_type = other DNA
ccaggcttcagcatctttgc

SEQ ID NO: 5 - DNA, 22 bp, synthetic construct
  source 1..22: mol_type = other DNA
tcatgatgctacccgaggtttg

SEQ ID NO: 6 - DNA, 22 bp, synthetic construct
  source 1..22: mol_type = other DNA
cagaactagatgcagccggaga

SEQ ID NO: 7 - DNA, 23 bp, synthetic construct
  source 1..23: mol_type = other DNA
tcgctcctcaagactgttcctcc

SEQ ID NO: 8 - DNA, 20 bp, synthetic construct
  source 1..20: mol_type = other DNA
caggcagtccctttacagca